European Patent Specification EP 3 778 621 B1, published August 23, 2023. Title: Peptide Synthesis Method. Applicant: Jitsubo Co., Ltd. The sequence listing filed with the application follows.

SEQUENCE LISTING (32 sequences)

SEQ ID NO: 1 - protein, 10 aa, Artificial Sequence
  Icatibant obtained by present peptide synthesis method
  MISC_FEATURE (1)..(1): X is D-Arg
  MISC_FEATURE (4)..(4): X is Hyp
  MISC_FEATURE (6)..(6): X is Thi
  MISC_FEATURE (8)..(8): X is D-Tic
  MISC_FEATURE (9)..(9): X is Oic
RRPXGXSXXR

SEQ ID NO: 2 - protein, 10 aa, Artificial Sequence
  leuprorelin
  MISC_FEATURE (1)..(1): X is Pyr
  MISC_FEATURE (6)..(6): X is D-Leu
  MISC_FEATURE (10)..(10): X is NHEt
XHWSYLLRPX

SEQ ID NO: 3 - protein, 8 aa, Artificial Sequence
  Peptide obtained by present peptide synthesis method, which is partial peptide of SEQ ID:2 having protective groups
  MISC_FEATURE (1)..(1): X is His(Trt)
  MISC_FEATURE (2)..(2): X is Trp(Boc)
  MISC_FEATURE (3)..(3): X is Ser(tBu)
  MISC_FEATURE (4)..(4): X is Tyr(tBu)
  MISC_FEATURE (5)..(5): X is D-Leu
  MISC_FEATURE (7)..(7): X is Arg(Pbf)
  MISC_FEATURE (8)..(8): X is OKb
HWSYLLRX

SEQ ID NO: 4 - protein, 9 aa, Artificial Sequence
  Peptide obtained by present peptide synthesis method, which is partial peptide of SEQ ID:2 having protective groups
  MISC_FEATURE (1)..(1): X is Pyr
  MISC_FEATURE (2)..(2): X is His(Trt)
  MISC_FEATURE (3)..(3): X is Trp(Boc)
  MISC_FEATURE (4)..(4): X is Ser(tBu)
  MISC_FEATURE (5)..(5): X is Tyr(tBu)
  MISC_FEATURE (6)..(6): X is D-Leu
  MISC_FEATURE (8)..(8): X is Arg(Pbf)
  MISC_FEATURE (9)..(9): X is OKb
XHWSYLLRX

SEQ ID NO: 5 - protein, 8 aa, Artificial Sequence
  Peptide obtained by present peptide synthesis method, which is partial peptide of SEQ ID:2 having protective groups
  MISC_FEATURE (1)..(1): X is Pyr
  MISC_FEATURE (2)..(2): X is His(Trt)
  MISC_FEATURE (3)..(2): X is Trp(Boc)
  MISC_FEATURE (4)..(4): X is Ser(tBu)
  MISC_FEATURE (5)..(5): X is Tyr(tBu)
  MISC_FEATURE (6)..(6): X is D-Leu
  MISC_FEATURE (8)..(8): X is Arg(Pbf)
XHWSYLLR

SEQ ID NO: 6 - protein, 10 aa, Artificial Sequence
  Peptide obtained by present peptide synthesis method, which is peptide of SEQ ID:2 having protective groups
  MISC_FEATURE (1)..(1): X is Pyr
  MISC_FEATURE (2)..(2): X is His(Trt)
  MISC_FEATURE (3)..(3): X is Trp(Boc)
  MISC_FEATURE (4)..(4): X is Ser(tBu)
  MISC_FEATURE (5)..(5): X is Tyr(tBu)
  MISC_FEATURE (6)..(6): X is D-Leu
  MISC_FEATURE (8)..(8): X is Arg(Pbf)
  MISC_FEATURE (10)..(10): X is NHEt
XHWSYLLRPX

SEQ ID NO: 7 - protein, 10 aa, Artificial Sequence
  Peptide obtained by present peptide synthesis method, which is partial peptide of SEQ ID:1 having protective groups
  MISC_FEATURE (1)..(1): X is Arg(Pbf)
  MISC_FEATURE (3)..(3): X is Hyp
  MISC_FEATURE (5)..(5): X is Thi
  MISC_FEATURE (6)..(6): X is Ser(tBu)
  MISC_FEATURE (7)..(7): X is D-Tic
  MISC_FEATURE (8)..(8): X is Oic
  MISC_FEATURE (9)..(9): X is Arg(Pbf)
  MISC_FEATURE (10)..(10): X is OKb
RPXGXSXXRX

SEQ ID NO: 8 - protein, 12 aa, Artificial Sequence
  Peptide obtained by present peptide synthesis method, which is peptide of SEQ ID:1 having protective groups
  MISC_FEATURE (1)..(1): X is Boc
  MISC_FEATURE (2)..(2): X is D-Arg(Pbf)
  MISC_FEATURE (3)..(3): X is Arg(Pbf)
  MISC_FEATURE (5)..(5): X is Hyp
  MISC_FEATURE (7)..(7): X is Thi
  MISC_FEATURE (8)..(8): X is Ser(tBu)
  MISC_FEATURE (9)..(9): X is D-Tic
  MISC_FEATURE (10)..(10): X is Oic
  MISC_FEATURE (11)..(11): X is Arg(Pbf)
  MISC_FEATURE (12)..(12): X is OKb
XRRPXGXSXXRX

SEQ ID NO: 9 - protein, 9 aa, Artificial Sequence
  Peptide obtained by present peptide synthesis method, which is partial peptide of SEQ ID:2 having protective groups
  MISC_FEATURE (1)..(1): X is His(Trt)
  MISC_FEATURE (2)..(2): X is Trp(Boc)
  MISC_FEATURE (3)..(3): X is Ser(tBu)
  MISC_FEATURE (4)..(4): X is Tyr(tBu)
  MISC_FEATURE (5)..(5): X is D-Leu
  MISC_FEATURE (7)..(7): X is Arg(Pbf)
  MISC_FEATURE (9)..(9): X is EtNKb
HWSYLLRPX

SEQ ID NO: 10 - protein, 10 aa, Artificial Sequence
  Peptide obtained by present peptide synthesis method, which is peptide of SEQ ID:2 having protective groups
  MISC_FEATURE (1)..(1): X is Pyr
  MISC_FEATURE (2)..(2): X is His(Trt)
  MISC_FEATURE (3)..(3): X is Trp(Boc)
  MISC_FEATURE (4)..(4): X is Ser(tBu)
  MISC_FEATURE (5)..(5): X is Tyr(tBu)
  MISC_FEATURE (6)..(6): X is D-Leu
  MISC_FEATURE (8)..(8): X is Arg(Pbf)
  MISC_FEATURE (10)..(10): X is EtNKb
XHWSYLLRPX

SEQ ID NO: 11 - protein, 4 aa, Artificial Sequence
  Synthetic peptide
  MISC_FEATURE (1)..(1): X is D-Tic
  MISC_FEATURE (2)..(2): X is Oic
  MISC_FEATURE (3)..(3): X is Arg(Pbf)
  MISC_FEATURE (4)..(4): X is OKa
XXRX

SEQ ID NO: 12 - protein, 5 aa, Artificial Sequence
  Peptide obtained by known peptide synthesis method, which is partial peptide of SEQ ID:1 having protective groups
  MISC_FEATURE (1)..(1): X is Ser(tBu)
  MISC_FEATURE (2)..(2): X is D-Tic
  MISC_FEATURE (3)..(3): X is Oic
  MISC_FEATURE (4)..(4): X is Arg(Pbf)
  MISC_FEATURE (5)..(5): X is OKa
SXXRX

SEQ ID NO: 13 - protein, 6 aa, Artificial Sequence
  Peptide obtained by known peptide synthesis method, which is partial peptide of SEQ ID:1 having protective groups
  MISC_FEATURE (1)..(1): X is Thi
  MISC_FEATURE (2)..(2): X is Ser(tBu)
  MISC_FEATURE (3)..(3): X is D-Tic
  MISC_FEATURE (4)..(4): X is Oic
  MISC_FEATURE (5)..(5): X is Arg(Pbf)
  MISC_FEATURE (6)..(6): X is OKa
XSXXRX

SEQ ID NO: 14 - protein, 7 aa, Artificial Sequence
  Peptide obtained by known peptide synthesis method, which is partial peptide of SEQ ID:1 having protective groups
  MISC_FEATURE (2)..(2): X is Thi
  MISC_FEATURE (3)..(3): X is Ser(tBu)
  MISC_FEATURE (4)..(4): X is D-Tic
  MISC_FEATURE (5)..(5): X is Oic
  MISC_FEATURE (6)..(6): X is Arg(Pbf)
  MISC_FEATURE (7)..(7): X is OKa
GXSXXRX

SEQ ID NO: 15 - protein, 8 aa, Artificial Sequence
  Peptide obtained by known peptide synthesis method, which is partial peptide of SEQ ID:1 having protective groups
  MISC_FEATURE (1)..(1): X is Hyp
  MISC_FEATURE (3)..(3): X is Thi
  MISC_FEATURE (4)..(4): X is Ser(tBu)
  MISC_FEATURE (5)..(5): X is D-Tic
  MISC_FEATURE (6)..(6): X is Oic
  MISC_FEATURE (7)..(7): X is Arg(Pbf)
  MISC_FEATURE (8)..(8): X is OKa
XGXSXXRX

SEQ ID NO: 16 - protein, 9 aa, Artificial Sequence
  Peptide obtained by known peptide synthesis method, which is partial peptide of SEQ ID:1 having protective groups
  MISC_FEATURE (2)..(2): X is Hyp
  MISC_FEATURE (4)..(4): X is Thi
  MISC_FEATURE (5)..(5): X is Ser(tBu)
  MISC_FEATURE (6)..(6): X is D-Tic
  MISC_FEATURE (7)..(7): X is Oic
  MISC_FEATURE (8)..(8): X is Arg(Pbf)
  MISC_FEATURE (9)..(9): X is OKa
PXGXSXXRX

SEQ ID NO: 17 - protein, 10 aa, Artificial Sequence
  Peptide obtained by known peptide synthesis method, which is partial peptide of SEQ ID:1 having protective groups
  MISC_FEATURE (1)..(1): X is Arg(Pbf)
  MISC_FEATURE (3)..(3): X is Hyp
  MISC_FEATURE (5)..(5): X is Thi
  MISC_FEATURE (6)..(6): X is Ser(tBu)
  MISC_FEATURE (7)..(7): X is D-Tic
  MISC_FEATURE (8)..(8): X is Oic
  MISC_FEATURE (9)..(9): X is Arg(Pbf)
  MISC_FEATURE (10)..(10): X is OKa
RPXGXSXXRX

SEQ ID NO: 18 - protein, 11 aa, Artificial Sequence
  Peptide obtained by known peptide synthesis method, which is peptide of SEQ ID:1 having protective groups
  MISC_FEATURE (1)..(1): X is D-Arg(Pbf)
  MISC_FEATURE (2)..(2): X is Arg(Pbf)
  MISC_FEATURE (4)..(4): X is Hyp
  MISC_FEATURE (6)..(6): X is Thi
  MISC_FEATURE (7)..(7): X is Ser(tBu)
  MISC_FEATURE (8)..(8): X is D-Tic
  MISC_FEATURE (9)..(9): X is Oic
  MISC_FEATURE (10)..(10): X is Arg(Pbf)
  MISC_FEATURE (11)..(11): X is OKa
RRPXGXSXXRX

SEQ ID NO: 19 - protein, 4 aa, Artificial Sequence
  Synthetic peptide, which is partial peptide of SEQ ID:2
  MISC_FEATURE (4)..(4): X is NHEt
LRPX

SEQ ID NO: 20 - protein, 4 aa, Artificial Sequence
  Synthetic peptide, which is partial peptide of SEQ ID:2 having protective group
  MISC_FEATURE (2)..(2): X is Arg(Pbf)
  MISC_FEATURE (4)..(4): X is NHEt
LRPX

SEQ ID NO: 21 - protein, 8 aa, Artificial Sequence
  Synthetic peptide, which is partial peptide of SEQ ID:2
  MISC_FEATURE (1)..(1): X is Pyr
  MISC_FEATURE (6)..(6): X is D-Leu
XHWSYLLR

SEQ ID NO: 22 - protein, 8 aa, Artificial Sequence
  Peptide obtained by present peptide synthesis method, which is partial peptide of SEQ ID:2 having protective groups
  MISC_FEATURE (1)..(1): X is His(Trt)
  MISC_FEATURE (2)..(2): X is Trp(Boc)
  MISC_FEATURE (3)..(3): X is Ser(tBu)
  MISC_FEATURE (4)..(4): X is Tyr(tBu)
  MISC_FEATURE (5)..(5): X is D-Leu
  MISC_FEATURE (7)..(7): X is Arg(Pbf)
  MISC_FEATURE (8)..(8): X is O-KS1
HWSYLLRX

SEQ ID NO: 23 - protein, 9 aa, Artificial Sequence
  Peptide obtained by present peptide synthesis method, which is partial peptide of SEQ ID:2 having protective groups
  MISC_FEATURE (1)..(1): X is Pyr
  MISC_FEATURE (2)..(2): X is His(Trt)
  MISC_FEATURE (3)..(3): X is Trp(Boc)
  MISC_FEATURE (4)..(4): X is Ser(tBu)
  MISC_FEATURE (5)..(5): X is Tyr(tBu)
  MISC_FEATURE (6)..(6): X is D-Leu
  MISC_FEATURE (8)..(8): X is Arg(Pbf)
  MISC_FEATURE (9)..(9): X is O-KS1
XHWSYLLRX

SEQ ID NO: 24 - protein, 8 aa, Artificial Sequence
  Peptide obtained by present peptide synthesis method, which is partial peptide of SEQ ID:2 having protective groups
  MISC_FEATURE (1)..(1): X is His(Trt)
  MISC_FEATURE (2)..(2): X is Trp(Boc)
  MISC_FEATURE (3)..(3): X is Ser(tBu)
  MISC_FEATURE (4)..(4): X is Tyr(tBu)
  MISC_FEATURE (5)..(5): X is D-Leu
  MISC_FEATURE (7)..(7): X is Arg(Pbf)
  MISC_FEATURE (8)..(8): X is O-Fl
HWSYLLRX

SEQ ID NO: 25 - protein, 9 aa, Artificial Sequence
  Peptide obtained by present peptide synthesis method, which is partial peptide of SEQ ID:2 having protective groups
  MISC_FEATURE (1)..(1): X is Pyr
  MISC_FEATURE (2)..(2): X is His(Trt)
  MISC_FEATURE (3)..(3): X is Trp(Boc)
  MISC_FEATURE (4)..(4): X is Ser(tBu)
  MISC_FEATURE (5)..(5): X is Tyr(tBu)
  MISC_FEATURE (6)..(6): X is D-Leu
  MISC_FEATURE (8)..(8): X is Arg(Pbf)
  MISC_FEATURE (9)..(9): X is O-Fl
XHWSYLLRX

SEQ ID NO: 26 - protein, 8 aa, Artificial Sequence
  Peptide obtained by present peptide synthesis method, which is partial peptide of SEQ ID:2 having protective groups
  MISC_FEATURE (1)..(1): X is His(Trt)
  MISC_FEATURE (2)..(2): X is Trp(Boc)
  MISC_FEATURE (3)..(3): X is Ser(tBu)
  MISC_FEATURE (4)..(4): X is Tyr(tBu)
  MISC_FEATURE (5)..(5): X is D-Leu
  MISC_FEATURE (7)..(7): X is Arg(Pbf)
  MISC_FEATURE (8)..(8): X is O-KJ1
HWSYLLRX

SEQ ID NO: 27 - protein, 9 aa, Artificial Sequence
  Peptide obtained by present peptide synthesis method, which is partial peptide of SEQ ID:2 having protective groups
  MISC_FEATURE (1)..(1): X is Pyr
  MISC_FEATURE (2)..(2): X is His(Trt)
  MISC_FEATURE (3)..(3): X is Trp(Boc)
  MISC_FEATURE (4)..(4): X is Ser(tBu)
  MISC_FEATURE (5)..(5): X is Tyr(tBu)
  MISC_FEATURE (6)..(6): X is D-Leu
  MISC_FEATURE (8)..(8): X is Arg(Pbf)
  MISC_FEATURE (9)..(9): X is O-KJ1
XHWSYLLRX

SEQ ID NO: 28 - protein, 9 aa, Artificial Sequence
  Peptide obtained by present peptide synthesis method, which is partial peptide of SEQ ID:2 having protective groups
  MISC_FEATURE (1)..(1): X is His(Trt)
  MISC_FEATURE (2)..(2): X is Trp(Boc)
  MISC_FEATURE (3)..(3): X is Ser(tBu)
  MISC_FEATURE (4)..(4): X is Tyr(tBu)
  MISC_FEATURE (5)..(5): X is D-Leu
  MISC_FEATURE (7)..(7): X is Arg(Pbf)
  MISC_FEATURE (9)..(9): X is NEt-KJ3
HWSYLLRPX

SEQ ID NO: 29 - protein, 10 aa, Artificial Sequence
  Peptide obtained by present peptide synthesis method, which is peptide of SEQ ID:2 having protective groups
  MISC_FEATURE (1)..(1): X is Pyr
  MISC_FEATURE (2)..(2): X is His(Trt)
  MISC_FEATURE (3)..(3): X is Trp(Boc)
  MISC_FEATURE (4)..(4): X is Ser(tBu)
  MISC_FEATURE (5)..(5): X is Tyr(tBu)
  MISC_FEATURE (6)..(6): X is D-Leu
  MISC_FEATURE (8)..(8): X is Arg(Pbf)
  MISC_FEATURE (10)..(10): X is NEt-KJ3
XHWSYLLRPX

SEQ ID NO: 30 - protein, 4 aa, Artificial Sequence
  Peptide obtained by present pepetide synthesis method, which is can be used in various fields
SPLQ

SEQ ID NO: 31 - protein, 4 aa, Artificial Sequence
  Peptide obtained by present peptide synthesis method, which is can be used in various fields
  MISC_FEATURE (3)..(3): X is Gln(Trt)
  MISC_FEATURE (4)..(4): X is OKb
PLQX

SEQ ID NO: 32 - protein, 6 aa, Artificial Sequence
  Peptide obtained by present peptide synthesis method, which is can be used in various fields
  MISC_FEATURE (1)..(1): X is Boc
  MISC_FEATURE (2)..(2): X is Ser(tBu)
  MISC_FEATURE (5)..(5): X is Gln(Trt)
  MISC_FEATURE (6)..(6): X is OKb
XSPLQX